European Patent Specification EP 2 817 625 B1, published January 1, 2025. Title: Chromatographic isolation of cells and other complex biological materials. Applicant: STAGE Cell Therapeutics GmbH. The sequence listing filed with the application follows.

SEQUENCE LISTING (13 sequences)

SEQ ID NO: 1 - protein, 253 aa, human
  Heavy Chain of Fab Fragment m13B8.2
AMQVQLKQSGPGLVQPSQSLSITCTVSGFSLTTFGVHWVRQSPGKGLEWLGVIWASGITDYNVPFMSRLSITKDNSKSQVFFKLNSLQPDDTAIYYCAKNDPGTGFAYWGQGTLVTVSAGSTKGPSVFPLAPSSKSTSGGTAALGCLVKDYFPEPVTVSWNSGALTSGVHTFPAVLQSSGLYSLSSVVTVPSSSLGTQTYICNVNHKPSNTKVDKKVEPKSCGSAWSHPQFEKGGGSGGGSGGSAWSHPQFEK

SEQ ID NO: 2 - protein, 218 aa, human
  Light Chain of Fab Fragment m13B8.2
AMDIQMTQSPASLSASVGETVTFTCRASEMIYSYLAWYQQKQGKSPQLLVHDAKTLAEGVPSRFSGGGSGTQFSLKINTLQPEDFGTYYCQAHYGNPPTFGGGTKLEIKRGIAAPSVFIFPPSDEQLKSGTASVVCLLNNFYPREAKVQWKVDNALQSGNSQESVTEQDSKDSTYSLSSTLTLSKADYEKHKVYACEVTHQGLSSPVTKSFNRGECGS

SEQ ID NO: 3 - protein, 8 aa, artificial
  streptavidin-binding peptide
WSHPQFEK

SEQ ID NO: 4 - protein, 9 aa, artificial
  HA-tag
YPYDVPDYA

SEQ ID NO: 5 - protein, 11 aa, artificial
  VSV-G.tag
YTDIEMNRLGK

SEQ ID NO: 6 - protein, 11 aa, artificial
  HSV-tag
QPELAPEDPED

SEQ ID NO: 7 - protein, 10 aa, artificial
  T7 epitope
ASMTGGQQMG

SEQ ID NO: 8 - protein, 10 aa, artificial
  myc-epitope
EQKLISEEDL

SEQ ID NO: 9 - protein, 14 aa, artificial
  V5-tag
GKPIPNPLLGLDST

SEQ ID NO: 10 - protein, 11 aa, artificial
  MAT-tag
HNHRHKHGGGC

SEQ ID NO: 11 - protein, 4 aa, artificial
  streptavidin mutein
VTAR

SEQ ID NO: 12 - protein, 4 aa, artificial
  streptavidin mutein analog
IGAR

SEQ ID NO: 13 - protein, 30 aa, artificial
  streptavidin binding module
SAWSHPQFEKGGGSGGGSGGSAWSHPQFEK